European Patent Specification EP 3 675 647 B1, published October 9, 2024. Title: ANIMAL FEED ADDITIVES COMPRISING POLYPEPTIDES HAVING PROTEASE ACTIVITY AND USES THEREOF. Applicant: Novozymes A/S. The sequence listing filed with the application follows.

SEQUENCE LISTING (10 sequences)

SEQ ID NO: 1 - protein, 314 aa, Bacillus horneckiae
  mat_peptide (1)..(314)
EVTATPSTQTPWGIKSIYNDQSITKTTGGSGIKVAVLDTGVHTGHIDLAGSSEQCKDFTQSNPLVNGSCTDRQGHGTHVAGTVLAHGGSDGQGVYGVAPQAKLWAYKVLGDNGSGYSDDIAAAIRHVADEASRTGSKVVINMSLGSSGKDSLIASAVDYAYGKGVLIVAAAGNSGSGSNTIGYPAALVNAVAVAALENVQQNGTYRVANFSSRGNPATAGDFRIQERDVEVSAPGASVESTWYNGGYNTISGTSMATPHVAGLAAKIWSSNSSLSHSQLRTELQNRAKVYDIKGGIGAGTGDDYASGFGYPRVK

SEQ ID NO: 2 - protein, 311 aa, Bacillus sp. [sequence omitted]

SEQ ID NO: 3 - protein, 311 aa, Artificial Sequence
  Protein Engineered variant
  mat_peptide (1)..(311)
AVPSTQTPWGIKSIYNDQSITKTTGGKGIKVAVLDTGVYTSHLDLAGSAEQCKDFTQSNPLVDGSCTDRQGHGTHVAGTVLAHGGSNGQGVYGVAPQAKLWAYKVLGDKGEGYSDDIAAAIRHVADEASRTGSKVVINMSLGSSAKDSLIASAVDYAYGKGVLIVAAAGNEGPKPNTIGYPAGFVNAVAVAALENVQEKGTYRVADFSSRGNPATAGDYIIQERDIEVSAPGASVESTWYTGGYNTISGTSMATPHVAGLAAKIWSANTSLSHSQLRTELQNRAKVYDIKGGIGAGPGDDYASGFGYPRVK

SEQ ID NO: 4 - protein, 12 aa, Artificial Sequence
  Conserved motif TGXKV[I/V]XXMSLG.
  MISC_FEATURE (3)..(3): The amino acid in position 3 is any amino acid.
  MISC_FEATURE (6)..(6): The amino acid in position 3 is valine (V) or isoleucine (I).
  MISC_FEATURE (7)..(7): The amino acid in position 7 is any amino acid.
  MISC_FEATURE (8)..(8): The amino acid in position 8 is any amino acid.
TGXKVXXXMSLG

SEQ ID NO: 5 - protein, 418 aa, Bacillus sp-13380
  PEPTIDE (1)..(418): Signal peptide: Residues 1-27
MKKKRIIGSAVLSVAMGLSVFASGAFGQQVESNETYRVVIQGPSAEKAKAKSNYGVRWDFGQKGFTTTVNAKQYQALLKNKNLKIDRVDEVKNAPVTAAKPGSGAASAPADGTPWGIEAIYNDSSIQSTSGGNGVKVAVLDTGVNTAHADLAGQAEQCKDFTQRKTPLIDGSCGDKNGHGTHVAGTVLAHGGANGQGVYGVAPDADLWAYKVLNDRGSGYSDDIAGAIKHAADEAVRTGSKVVISMSLGSSSKSTLIADAVDYAYSKGVLVVAAAGNDGPADNTIGYPGALVNAVAVAALENVQQNGSYRVADFSSRGNPATDGDFVIQERDVEVSAPGRAIESTWYDGSYSTISGTSMATPHVSGLAAKIWAQNPSMSHTQLRAELQSRAKQNDILGGTGAAAGDDYASGFGFPRVK

SEQ ID NO: 6 - protein, 417 aa, Bacillus idriensis
  PEPTIDE (1)..(417): Signal peptide: Residues 1-27
MKIRKVLGVAVLSLSMSLSMFGTNTFAQDAAKTDVNQDSIRVVIKGTDTEKVKMKKSHKVRRDFGKDGFTTTVNAKEYEALIKNDKIKVEKVSTLQVAAGKPIKTMALPSTRTPWGIKAIYNNSSLTSTSGGDGIKIAVLDTGVQTSHIDLSQNVEQCKDFTVGSSYTNGSCTDRNGHGTHVAGTALANGGSDGMGIYGVAPQSELWAYKVLTDSGSGYSDDIAAAIRHAADEGTRTGSKVIISMSLGSSGKDSLIASAVDYAYGKGALVIAAAGNSGSGNNTIGYPGALVNAVAVAALENVQQNGTYRVANFSSRGNSATDGDFIIGERDVEISAPGASIESTWINSGYNTISGTSMATPHVSGLAAKIWSSNKSQSNVQVRAELQNRAKLYDIKGGIGAATGDDHASGFGFARVQ

SEQ ID NO: 7 - protein, 413 aa, Bacillus sp
  PEPTIDE (1)..(413): Signal peptide: Residues 1-27
LLSMTMGLSVFTAGAFAKEPETQNETYRVLIQGPANAKASVNSQVDKRWDFGSDGMTAEVNAKQYQALLKNKNLKIEKVSEVTLDTARTEASKKDSVSIQAAGYPSDQTPWGIASIYNNSSITSTSGGSGIKVAVLDTGVYTGHIDLEGSAEQCKDFTQSTPLVNGSCTDRQGHGTHVAGTVLAHGGYDGQGIYGVAPQAKLWAYKVLGDNGSGYSDDIAGAIRHVADEASRTGSKVVINMSLGSSGKDSLISSAVDYAYSKGVLVVAAAGNSGYSANTIGYPGALKNAIAVAALENVQQNGTYRVANFSSRGNPNTDGDYIIQEKDVEVSAPGASIESTWYNGGYNTISGTSMATPHVAGLAAKIWSSSPSMSHTQLRTELQNRAKQYDIKGGYGAATGDDYASGFGYPRVK

SEQ ID NO: 8 - protein, 420 aa, Bacillus sp
  PEPTIDE (1)..(420): Signal peptide: Residues 1-29
MTKKKTVAAALLSLTLGMSVFTSGISAQVSDEAKGSETYRVLIQAPSNSVNALETKYEKRWDFGKEGFTADVNAKELQTLQATKNVEVQKVNEMSIATVTGEVSKAEVTAVPSSQTPWGIKSIYNNQSLTATSGGNGIKVAVLDTGVYTNHIDLAGSAEQCKDFTQSSPLVNGSCTDRQGHGTHVAGTVLAHGGSDGQGVYGVAPDAKLWAYKVLGDNGSGYSDDIAAAIRHVADQATSTGSKVVINMSLGSSGKDSLISSAVDYAYNKGVLVVAAAGNSGSGSNTIGYPGALVNAVAVAALENVQQNGTYRVANFSSRGNPSTDGDYVIQERDIEVSAPGAAVESTWYNGGYNTISGTSMATPHVAGLAAKIWASNPSWSKSTLRTELQNRAKVYDIKGGVGATTGDDYASGFGYPRVK

SEQ ID NO: 9 - protein, 425 aa, Bacillus oceanisediminis
  PEPTIDE (1)..(425): Signal peptide: Residues 1-25
MKKKRVLGAALLSMTMGLSVFTAGAFAKGPEANESYRVLIQGPAAERANVKAQIEERWDFGKDGLTAEVNSKQYQALLKNKNITIEKVSEVTLDTARTEASSSKNDSISLEAAGYPSDQTPWGIESIYNNSYISSTSGGSGIKVAVLDTGVYTNHIDLEGSAEQCKDFTQSYSSMVNGTCTDRQGHGTHVAGTVLAHGGYDGLGVYGVAPQAKLWAYKVLGDNGSGYSDDIAGAIRHVADEAVRTGSKVVINMSLGSSGKDSLIASAVDYAYSKGVLIVAAAGNSGYSANTIGYPGALTNAIAVAALENVQQNGTYRVANFSSRGNPNTDGDYYIQERDVEVSAPGASIESTWYNGGYNTISGTSMATPHVAGLAAKIWSSNPYMSHTQLRTELRNRAKQYDIKGGYGAATGDDYASGFGYPRVR

SEQ ID NO: 10 - DNA, 1278 bp, Bacillus oceanisediminis
atgaagaagaagcgcgtacttggcgcagctcttctttcaatgacaatgggcctttcagtattcacagctggcgcatttgctaaaggtcctgaggctaacgagtcttaccgcgtacttatccaaggacctgcggctgaacgcgctaacgttaaagcccaaatcgaggagcgctgggactttggtaaagacggtcttacggctgaggttaactctaaacagtaccaggctcttcttaagaacaaaaacatcactatcgagaaagtttcagaggttacgttagacacagctcgcactgaggcttcatcaagcaaaaacgactcaatctcacttgaggcagctggctatccttcagaccaaactccttggggcatcgagtcaatctacaacaactcttacatctcatcaacatcaggaggctcaggtatcaaagttgcagttttagacactggcgtttacacaaaccacatcgaccttgagggctctgcagagcagtgcaaagactttactcagtcttactcatcaatggttaacggtacgtgcacagaccgccagggccatggcacacacgtagcaggcacagttcttgcgcacggtggctacgacggccttggtgtatatggcgttgcacctcaagccaaactttgggcttacaaagttcttggcgacaacggatcaggctattcagacgacatcgcaggcgctatccgccacgtagctgacgaggctgttcgcacaggatcaaaagtagtaatcaacatgtcacttggaagctcaggtaaagactcacttatcgcgtcagctgttgactatgcttattcaaaaggcgttcttatcgttgctgcggctggtaactcaggttattcagcaaacacaatcggctaccctggtgcgcttacgaacgcaatcgctgttgccgctcttgagaacgtacaacagaacggcacttatcgcgttgcgaacttttcatcacgcggaaaccctaacacagacggcgactactatatccaggagcgcgacgttgaggtttcagctcctggtgcttcaatcgagtcaacgtggtacaatggtggctacaacactatctcaggcacgtcaatggctacgcctcacgttgctggccttgctgcgaaaatctggtcttcaaacccttacatgtcacacactcaacttcgcactgagcttcgcaatcgcgctaaacaatacgacatcaaaggtggatatggagctgctactggtgacgactacgcatcaggttttggttatcctcgcgttcgctaa